European Patent Application EP 4 810 520 A1, published September 23, 2026. Title: 一种抗PD-1抗体及其生物材料和产品. Applicant: 成都盛世君联生物技术有限公司. Application CN. The sequence listing filed with the application follows.

SEQUENCE LISTING (72 sequences)

SEQ ID NO: 1 - protein, 5 aa, synthetic construct
IELMA

SEQ ID NO: 2 - protein, 15 aa, synthetic construct
GISADTQNVEDSLEG

SEQ ID NO: 3 - protein, 17 aa, synthetic construct
RGYNMRNPNVGRLPYDA

SEQ ID NO: 4 - protein, 30 aa, synthetic construct
QVQLVESGGGVVQVGGSLRLSCTASGNDFS

SEQ ID NO: 5 - protein, 14 aa, synthetic construct
WYRQAPGKEREWVA

SEQ ID NO: 6 - protein, 32 aa, synthetic construct
RFTISRDSTKNTVYLQMNSLKPEDTALYRCNV

SEQ ID NO: 7 - protein, 11 aa, synthetic construct
WGQGTQVTVSS

SEQ ID NO: 8 - protein, 5 aa, synthetic construct
PKTMA

SEQ ID NO: 9 - protein, 17 aa, synthetic construct
SIYTTTGITYYTDSVQG

SEQ ID NO: 10 - protein, 17 aa, synthetic construct
ALTEIGRYRLYARQYDF

SEQ ID NO: 11 - protein, 30 aa, synthetic construct
QVKLVESGGGSVQAGGSLRLSCARANFASS

SEQ ID NO: 12 - protein, 14 aa, synthetic construct
WFRQAPGKEREGVA

SEQ ID NO: 13 - protein, 32 aa, synthetic construct
RFSISQDMAKNTVYLQMNSLKPEDTAMYYCAA

SEQ ID NO: 14 - protein, 11 aa, synthetic construct
WGQGTQVTVSS

SEQ ID NO: 15 - protein, 5 aa, synthetic construct
AADMG

SEQ ID NO: 16 - protein, 17 aa, synthetic construct
AILTGVGTIYYADSLKG

SEQ ID NO: 17 - protein, 14 aa, synthetic construct
RPFGCNWRFYEYNY

SEQ ID NO: 18 - protein, 30 aa, synthetic construct
EVQLVESGGGSVEAGGSLTLSCLASGMNFD

SEQ ID NO: 19 - protein, 14 aa, synthetic construct
WYRQLPGNECEGVA

SEQ ID NO: 20 - protein, 32 aa, synthetic construct
RFTISQDNAKNTVYLQMNSLKPEDTAMYYCAA

SEQ ID NO: 21 - protein, 11 aa, synthetic construct
WGQGTQVTVSS

SEQ ID NO: 22 - protein, 5 aa, synthetic construct
DYAIG

SEQ ID NO: 23 - protein, 17 aa, synthetic construct
CIAKTDGSTFYAHFAKD

SEQ ID NO: 24 - protein, 16 aa, synthetic construct
LHDCHPAGTRVSLTGS

SEQ ID NO: 25 - protein, 30 aa, synthetic construct
QVQLVESGGGLVQAGGSLRLTCAATGTGAD

SEQ ID NO: 26 - protein, 14 aa, synthetic construct
WFRQVPGVEREGVS

SEQ ID NO: 27 - protein, 32 aa, synthetic construct
RFTISRDNAKNAVYLQMNSLKPEDTGVYYCAL

SEQ ID NO: 28 - protein, 11 aa, synthetic construct
WGPGTRVTVSS

SEQ ID NO: 29 - protein, 5 aa, synthetic construct
DYAVG

SEQ ID NO: 30 - protein, 18 aa, synthetic construct
CIEKSPNVDTYYAIFAKD

SEQ ID NO: 31 - protein, 16 aa, synthetic construct
LHYCPNAGTRVSLKGS

SEQ ID NO: 32 - protein, 30 aa, synthetic construct
QVQLVESGGGLVQAGGSLRLSCTAGGFKFD

SEQ ID NO: 33 - protein, 14 aa, synthetic construct
WVRQAPGKEREGVA

SEQ ID NO: 34 - protein, 32 aa, synthetic construct
RFTISRNDAQTTVYLQMNSLKVEDTALYHCAM

SEQ ID NO: 35 - protein, 11 aa, synthetic construct
WGPGTQVTVSS

SEQ ID NO: 36 - protein, 5 aa, synthetic construct
NNCMG

SEQ ID NO: 37 - protein, 18 aa, synthetic construct
GIHTGRPSQQSYADSVKD

SEQ ID NO: 38 - protein, 19 aa, synthetic construct
RPGGQKYDCYSGSWYRSGY

SEQ ID NO: 39 - protein, 30 aa, synthetic construct
QVKLVESGGGSVQAGGSLRLSCAAPGYLYS

SEQ ID NO: 40 - protein, 14 aa, synthetic construct
WFRQAPGKEREWVV

SEQ ID NO: 41 - protein, 32 aa, synthetic construct
RFTISEDSAKNTVYLQMNSLKPEDTAMYYCAA

SEQ ID NO: 42 - protein, 11 aa, synthetic construct
WGQGTQVTVSS

SEQ ID NO: 43 - protein, 5 aa, synthetic construct
SYAMT

SEQ ID NO: 44 - protein, 18 aa, synthetic construct
AISSGDGVFTEYADSVKG

SEQ ID NO: 45 - protein, 8 aa, synthetic construct
GGYETYDG

SEQ ID NO: 46 - protein, 30 aa, synthetic construct
QVQLVQSGGGLVQPGGSLRLSCAASGFTFS

SEQ ID NO: 47 - protein, 14 aa, synthetic construct
WVRQTPGKGLEWVA

SEQ ID NO: 48 - protein, 32 aa, synthetic construct
RFTISRDNAKNTLYLQLNSLKTEDTAMYYCAK

SEQ ID NO: 49 - protein, 11 aa, synthetic construct
RGQGTQVTVSS

SEQ ID NO: 50 - protein, 5 aa, synthetic construct
DFDVG

SEQ ID NO: 51 - protein, 16 aa, synthetic construct
TISSDGRTYYEDSVKG

SEQ ID NO: 52 - protein, 20 aa, synthetic construct
NPHFIAMSGPCTVVRRGMDY

SEQ ID NO: 53 - protein, 30 aa, synthetic construct
EVKLVESGGGSVNTGGSLRLSCTSSGFTFD

SEQ ID NO: 54 - protein, 14 aa, synthetic construct
WYRQVRRDECELVS

SEQ ID NO: 55 - protein, 32 aa, synthetic construct
RFDISQDNAKNTVYLQMNRLAPEDAAVYYCAA

SEQ ID NO: 56 - protein, 11 aa, synthetic construct
WGKGTLVTISS

SEQ ID NO: 57 - protein, 5 aa, synthetic construct
SYAMT

SEQ ID NO: 58 - protein, 18 aa, synthetic construct
AISSGDGVFTEYADSVKG

SEQ ID NO: 59 - protein, 9 aa, synthetic construct
LGTRGWYLD

SEQ ID NO: 60 - protein, 30 aa, synthetic construct
QVQLVESGGGLVQPGGSLRLSCAASGFTFS

SEQ ID NO: 61 - protein, 14 aa, synthetic construct
WVRQTPGKGLEWVA

SEQ ID NO: 62 - protein, 32 aa, synthetic construct
RFTISRDNAKNTLYLQLNSLKTEDTAMYYCAR

SEQ ID NO: 63 - protein, 11 aa, synthetic construct
WGQGTQVTVSS

SEQ ID NO: 64 - protein, 125 aa, synthetic construct
QVQLVESGGGLVQAGGSLRLTCAATGTGADDYAIGWFRQVPGVEREGVSCIAKTDGSTFYAHFAKDRFTISRDNAKNAVYLQMNSLKPEDTGVYYCALLHDCHPAGTRVSLTGSWGPGTRVTVSS

SEQ ID NO: 65 - protein, 124 aa, synthetic construct
QVQLVESGGGVVQVGGSLRLSCTASGNDFSIELMAWYRQAPGKEREWVAGISADTQNVEDSLEGRFTISRDSTKNTVYLQMNSLKPEDTALYRCNVRGYNMRNPNVGRLPYDAWGQGTQVTVSS

SEQ ID NO: 66 - protein, 126 aa, synthetic construct
QVQLVESGGGLVQAGGSLRLSCTAGGFKFDDYAVGWVRQAPGKEREGVACIEKSPNVDTYYAIFAKDRFTISRNDAQTTVYLQMNSLKVEDTALYHCAMLHYCPNAGTRVSLKGSWGPGTQVTVSS

SEQ ID NO: 67 - protein, 126 aa, synthetic construct
QVKLVESGGGSVQAGGSLRLSCARANFASSPKTMAWFRQAPGKEREGVASIYTTTGITYYTDSVQGRFSISQDMAKNTVYLQMNSLKPEDTAMYYCAAALTEIGRYRLYARQYDFWGQGTQVTVSS

SEQ ID NO: 68 - protein, 129 aa, synthetic construct
QVKLVESGGGSVQAGGSLRLSCAAPGYLYSNNCMGWFRQAPGKEREWVVGIHTGRPSQQSYADSVKDRFTISEDSAKNTVYLQMNSLKPEDTAMYYCAARPGGQKYDCYSGSWYRSGYWGQGTQVTVSS

SEQ ID NO: 69 - protein, 118 aa, synthetic construct
QVQLVQSGGGLVQPGGSLRLSCAASGFTFSSYAMTWVRQTPGKGLEWVAAISSGDGVFTEYADSVKGRFTISRDNAKNTLYLQLNSLKTEDTAMYYCAKGGYETYDGRGQGTQVTVSS

SEQ ID NO: 70 - protein, 128 aa, synthetic construct
EVKLVESGGGSVNTGGSLRLSCTSSGFTFDDFDVGWYRQVRRDECELVSTISSDGRTYYEDSVKGRFDISQDNAKNTVYLQMNRLAPEDAAVYYCAANPHFIAMSGPCTVVRRGMDYWGKGTLVTISS

SEQ ID NO: 71 - protein, 119 aa, synthetic construct
QVQLVESGGGLVQPGGSLRLSCAASGFTFSSYAMTWVRQTPGKGLEWVAAISSGDGVFTEYADSVKGRFTISRDNAKNTLYLQLNSLKTEDTAMYYCARLGTRGWYLDWGQGTQVTVSS

SEQ ID NO: 72 - protein, 123 aa, synthetic construct
EVQLVESGGGSVEAGGSLTLSCLASGMNFDAADMGWYRQLPGNECEGVAAILTGVGTIYYADSLKGRFTISQDNAKNTVYLQMNSLKPEDTAMYYCAARPFGCNWRFYEYNYWGQGTQVTVSS